European Patent Application EP 4 556 560 A1, published May 21, 2025. Title: Mutant microorganism of Corynebacterium genus producing L-glutamic acid and method for producing L-glutamic acid using the same. Applicant: DAESANG CORPORATION. The sequence listing filed with the application follows.

SEQUENCE LISTING (9 sequences)

SEQ ID NO: 1 - DNA, 1503 bp, synthetic construct
  source 1..1503: mol_type = other DNA
atgtcagattccccgaagaacgcaccgaggattaccgatgaggcagatgtagttctcattggtgccggtatcatgagctccacgctgggtgcaatgctgcgtcagctggagccaagctggactcagatcgtcttcgagcgtttggatggaccggcacaagagtcgtcctccccgtggaacaatgcaggaaccggccactctgctctatgcgagctgaactacaccccagaggttaagggcaaggttgaaattgccaaggctgtaggaatcaacgagaagttccaggtttcccgtcagttctggtctcacctcgttgaagagggcgtgctggctgattctaaggaattcatcaaccctgttcctcacgtatctttcggccagggcgcagaccaggttgcatacatcaaggctcgctacgaagctttgaaggatcacccactcttccagggcatgacctacgctgacgatgaagctaccttcaccgagaagctgcctttgatggcaaagggccgtgacttctctgatccagtagcaatctcttggatcgatgaaggcaccgacatcaactacggtgctcagaccaagcagtacctggatgcatctgaagttgaaggcactgaaatccgctatggccacgaagtcaagagcatcaaggctgatggcgcaaagtggatcgtgaccgtcaagaacgtacacactggcgacaccaagaccatcaaggcaaacttcgtgttcgtcggcgcaggcgggtacgcactggatctgcttcgcagcgcaggcatcccacaggtcaagggcttcgctggattcccagtatccggcctgtggcttcgttgcaccaacgaggaactgatcgagcagcacgcagccaaggtatatggcaaggcatctgttggcgctcctccaatgtctgttcctcaccttgacacccgcgttatcgagggtgaaaagggtctgctctttggaccttacggtggctggacccctaagttcttgaaggaaggctcctacctggacctgttcaagtccatccgcccagacaacattccttcctaccttggcgttgctgctcaggaatttgatctgaccaagtaccttgtcactgaagttctcaaggaccaggacaagcgtatggatgctcttcgcgagtacatgccagaggcacaaaacggcgattgggagaccatcgttgccggacagcgtgttcaggttattaagcctgcaggattccctaagttcggttccctggaattcggcaccaccttgatcaacaactccgaaggcaccatcgccggattgctcggtgcttcccctggagcatccatcgcaccttccgcaatgatcgagctgcttgagcgttgcttcggtgaccgcatgatcgagtggggcgacaagctgaaggacatgatcccttcctacggcaagaagcttgcttccgagccagcactgtttgagcagcagtgggcacgcacccagaagaccctgaagcttgaggaagcctaa

SEQ ID NO: 2 - protein, 500 aa, synthetic construct
MSDSPKNAPRITDEADVVLIGAGIMSSTLGAMLRQLEPSWTQIVFERLDGPAQESSSPWNNAGTGHSALCELNYTPEVKGKVEIAKAVGINEKFQVSRQFWSHLVEEGVLADSKEFINPVPHVSFGQGADQVAYIKARYEALKDHPLFQGMTYADDEATFTEKLPLMAKGRDFSDPVAISWIDEGTDINYGAQTKQYLDASEVEGTEIRYGHEVKSIKADGAKWIVTVKNVHTGDTKTIKANFVFVGAGGYALDLLRSAGIPQVKGFAGFPVSGLWLRCTNEELIEQHAAKVYGKASVGAPPMSVPHLDTRVIEGEKGLLFGPYGGWTPKFLKEGSYLDLFKSIRPDNIPSYLGVAAQEFDLTKYLVTEVLKDQDKRMDALREYMPEAQNGDWETIVAGQRVQVIKPAGFPKFGSLEFGTTLINNSEGTIAGLLGASPGASIAPSAMIELLERCFGDRMIEWGDKLKDMIPSYGKKLASEPALFEQQWARTQKTLKLEEA

SEQ ID NO: 3 - DNA, 1503 bp, Corynebacterium sp.
  source 1..1503: mol_type = genomic DNA
atgtcagattccccgaagaacgcaccgaggattaccgatgaggcagatgtagttctcattggtgccggtatcatgagctccacgctgggtgcaatgctgcgtcagctggagccaagctggactcagatcgtcttcgagcgtttggatggaccggcacaagagtcgtcctccccgtggaacaatgcaggaaccggccactctgctctatgcgagctgaactacaccccagaggttaagggcaaggttgaaattgccaaggctgtaggaatcaacgagaagttccaggtttcccgtcagttctggtctcacctcgttgaagagggcgtgctggctgatcctaaggaattcatcaaccctgttcctcacgtatctttcggccagggcgcagaccaggttgcatacatcaaggctcgctacgaagctttgaaggatcacccactcttccagggcatgacctacgctgacgatgaagctaccttcaccgagaagctgcctttgatggcaaagggccgtgacttctctgatccagtagcaatctcttggatcgatgaaggcaccgacatcaactacggtgctcagaccaagcagtacctggatgcatctgaagttgaaggcactgaaatccgctatggccacgaagtcaagagcatcaaggctgatggcgcaaagtggatcgtgaccgtcaagaacgtacacactggcgacaccaagaccatcaaggcaaacttcgtgttcgtcggcgcaggcgggtacgcactggatctgcttcgcagcgcaggcatcccacaggtcaagggcttcgctggattcccagtatccggcctgtggcttcgttgcaccaacgaggaactgatcgagcagcacgcagccaaggtatatggcaaggcatctgttggcgctcctccaatgtctgttcctcaccttgacacccgcgttatcgagggtgaaaagggtctgctctttggaccttacggtggctggacccctaagttcttgaaggaaggctcctacctggacctgttcaagtccatccgcccagacaacattccttcctaccttggcgttgctgctcaggaatttgatctgaccaagtaccttgtcactgaagttctcaaggaccaggacaagcgtatggatgctcttcgcgagtacatgccagaggcacaaaacggcgattgggagaccatcgttgccggacagcgtgttcaggttattaagcctgcaggattccctaagttcggttccctggaattcggcaccaccttgatcaacaactccgaaggcaccatcgccggattgctcggtgcttcccctggagcatccatcgcaccttccgcaatgatcgagctgcttgagcgttgcttcggtgaccgcatgatcgagtggggcgacaagctgaaggacatgatcccttcctacggcaagaagcttgcttccgagccagcactgtttgagcagcagtgggcacgcacccagaagaccctgaagcttgaggaagcctaa

SEQ ID NO: 4 - protein, 500 aa, Corynebacterium sp.
MSDSPKNAPRITDEADVVLIGAGIMSSTLGAMLRQLEPSWTQIVFERLDGPAQESSSPWNNAGTGHSALCELNYTPEVKGKVEIAKAVGINEKFQVSRQFWSHLVEEGVLADPKEFINPVPHVSFGQGADQVAYIKARYEALKDHPLFQGMTYADDEATFTEKLPLMAKGRDFSDPVAISWIDEGTDINYGAQTKQYLDASEVEGTEIRYGHEVKSIKADGAKWIVTVKNVHTGDTKTIKANFVFVGAGGYALDLLRSAGIPQVKGFAGFPVSGLWLRCTNEELIEQHAAKVYGKASVGAPPMSVPHLDTRVIEGEKGLLFGPYGGWTPKFLKEGSYLDLFKSIRPDNIPSYLGVAAQEFDLTKYLVTEVLKDQDKRMDALREYMPEAQNGDWETIVAGQRVQVIKPAGFPKFGSLEFGTTLINNSEGTIAGLLGASPGASIAPSAMIELLERCFGDRMIEWGDKLKDMIPSYGKKLASEPALFEQQWARTQKTLKLEEA

SEQ ID NO: 5 - DNA, 5719 bp, synthetic construct
  source 1..5719: mol_type = other DNA
tgccgcaagcactcagggcgcaagggctgctaaaggaagcggaacacgtagaaagccagtccgcagaaacggtgctgaccccggatgaatgtcagctactgggctatctggacaagggaaaacgcaagcgcaaagagaaagcaggtagcttgcagtgggcttacatggcgatagctagactgggcggttttatggacagcaagcgaaccggaattgccagctggggcgccctctggtaaggttgggaagccctgcaaagtaaactggatggctttcttgccgccaaggatctgatggcgcaggggatcaagatctgatcaagagacaggatgaggatcgtttcgcatgattgaacaagatggattgcacgcaggttctccggccgcttgggtggagaggctattcggctatgactgggcacaacagacaatcggctgctctgatgccgccgtgttccggctgtcagcgcaggggcgcccggttctttttgtcaagaccgacctgtccggtgccctgaatgaactccaagacgaggcagcgcggctatcgtggctggccacgacgggcgttccttgcgcagctgtgctcgacgttgtcactgaagcgggaagggactggctgctattgggcgaagtgccggggcaggatctcctgtcatctcaccttgctcctgccgagaaagtatccatcatggctgatgcaatgcggcggctgcatacgcttgatccggctacctgcccattcgaccaccaagcgaaacatcgcatcgagcgagcacgtactcggatggaagccggtcttgtcgatcaggatgatctggacgaagagcatcaggggctcgcgccagccgaactgttcgccaggctcaaggcgcggatgcccgacggcgaggatctcgtcgtgacccatggcgatgcctgcttgccgaatatcatggtggaaaatggccgcttttctggattcatcgactgtggccggctgggtgtggcggaccgctatcaggacatagcgttggctacccgtgatattgctgaagagcttggcggcgaatgggctgaccgcttcctcgtgctttacggtatcgccgctcccgattcgcagcgcatcgccttctatcgccttcttgacgagttcttctgagcgggactctggggttcgctagaggatcgatcctttttaacccatcacatatacctgccgttcactattatttagtgaaatgagatattatgatattttctgaattgtgattaaaaaggcaactttatgcccatgcaacagaaactataaaaaatacagagaatgaaaagaaacagatagattttttagttctttaggcccgtagtctgcaaatccttttatgattttctatcaaacaaaagaggaaaatagaccagttgcaatccaaacgagagtctaatagaatgaggtcgaaaagtaaatcgcgcgggtttgttactgataaagcaggcaagacctaaaatgtgtaaagggcaaagtgtatactttggcgtcaccccttacatattttaggtctttttttattgtgcgtaactaacttgccatcttcaaacaggagggctggaagaagcagaccgctaacacagtacataaaaaaggagacatgaacgatgaacatcaaaaagtttgcaaaacaagcaacagtattaacctttactaccgcactgctggcaggaggcgcaactcaagcgtttgcgaaagaaacgaaccaaaagccatataaggaaacatacggcatttcccatattacacgccatgatatgctgcaaatccctgaacagcaaaaaaatgaaaaatatcaagtttctgaatttgattcgtccacaattaaaaatatctcttctgcaaaaggcctggacgtttgggacagctggccattacaaaacgctgacggcactgtcgcaaactatcacggctaccacatcgtctttgcattagccggagatcctaaaaatgcggatgacacatcgatttacatgttctatcaaaaagtcggcgaaacttctattgacagctggaaaaacgctggccgcgtctttaaagacagcgacaaattcgatgcaaatgattctatcctaaaagaccaaacacaagaatggtcaggttcagccacatttacatctgacggaaaaatccgtttattctacactgatttctccggtaaacattacggcaaacaaacactgacaactgcacaagttaacgtatcagcatcagacagctctttgaacatcaacggtgtagaggattataaatcaatctttgacggtgacggaaaaacgtatcaaaatgtacagcagttcatcgatgaaggcaactacagctcaggcgacaaccatacgctgagagatcctcactacgtagaagataaaggccacaaatacttagtatttgaagcaaacactggaactgaagatggctaccaaggcgaagaatctttatttaacaaagcatactatggcaaaagcacatcattcttccgtcaagaaagtcaaaaacttctgcaaagcgataaaaaacgcacggctgagttagcaaacggcgctctcggtatgattgagctaaacgatgattacacactgaaaaaagtgatgaaaccgctgattgcatctaacacagtaacagatgaaattgaacgcgcgaacgtctttaaaatgaacggcaaatggtacctgttcactgactcccgcggatcaaaaatgacgattgacggcattacgtctaacgatatttacatgcttggttatgtttctaattctttaactggcccatacaagccgctgaacaaaactggccttgtgttaaaaatggatcttgatcctaacgatgtaacctttacttactcacacttcgctgtacctcaagcgaaaggaaacaatgtcgtgattacaagctatatgacaaacagaggattctacgcagacaaacaatcaacgtttgcgccgagcttcctgctgaacatcaaaggcaagaaaacatctgttgtcaaagacagcatccttgaacaaggacaattaacagttaacaaataaaaacgcaaaagaaaatgccgatgggtaccgagcgaaatgaccgaccaagcgacgcccaacctgccatcacgagatttcgattccaccgccgccttctatgaaaggttgggcttcggaatcgttttccgggacgccctcgcggacgtgctcatagtccacgacgcccgtgattttgtagccctggccgacggccagcaggtaggccgacaggctcatgccggccgccgccgccttttcctcaatcgctcttcgttcgtctggaaggcagtacaccttgataggtgggctgcccttcctggttggcttggtttcatcagccatccgcttgccctcatctgttacgccggcggtagccggccagcctcgcagagcaggattcccgttgagcaccgccaggtgcgaataagggacagtgaagaaggaacacccgctcgcgggtgggcctacttcacctatcctgcccggctgacgccgttggatacaccaaggaaagtctacacgaaccctttggcaaaatcctgtatatcgtgcgaaaaaggatggatataccgaaaaaatcgctataatgaccccgaagcagggttatgcagcggaaaagcgctgcttccctgctgttttgtggaatatctaccgactggaaacaggcaaatgcaggaaattactgaactgaggggacaggcgagagacgatgccaaagagctcctgaaaatctcgataactcaaaaaatacgcccggtagtgatcttatttcattatggtgaaagttggaacctcttacgtgccgatcaacgtctcattttcgccaaaagttggcccagggcttcccggtatcaacagggacaccaggatttatttattctgcgaagtgatcttccgtcacaggtatttattcggcgcaaagtgcgtcgggtgatgctgccaacttactgatttagtgtatgatggtgtttttgaggtgctccagtggcttctgtttctatcagctcctgaaaatctcgataactcaaaaaatacgcccggtagtgatcttatttcattatggtgaaagttggaacctcttacgtgccgatcaacgtctcattttcgccaaaagttggcccagggcttcccggtatcaacagggacaccaggatttatttattctgcgaagtgatcttccgtcacaggtatttattcggcgcaaagtgcgtcgggtgatgctgccaacttactgatttagtgtatgatggtgtttttgaggtgctccagtggcttctgtttctatcagggctggatgatcctccagcgcggggatctcatgctggagttcttcgcccaccccaaaaggatctaggtgaagatcctttttgataatctcatgaccaaaatcccttaacgtgagttttcgttccactgagcgtcagaccccgtagaaaagatcaaaggatcttcttgagatcctttttttctgcgcgtaatctgctgcttgcaaacaaaaaaaccaccgctaccagcggtggtttgtttgccggatcaagagctaccaactctttttccgaaggtaactggcttcagcagagcgcagataccaaatactgttcttctagtgtagccgtagttaggccaccacttcaagaactctgtagcaccgcctacatacctcgctctgctaatcctgttaccagtggctgctgccagtggcgataagtcgtgtcttaccgggttggactcaagacgatagttaccggataaggcgcagcggtcgggctgaacggggggttcgtgcacacagcccagcttggagcgaacgacctacaccgaactgagatacctacagcgtgagctatgagaaagcgccacgcttcccgaagggagaaaggcggacaggtatccggtaagcggcagggtcggaacaggagagcgcacgagggagcttccagggggaaacgcctggtatctttatagtcctgtcgggtttcgccacctctgacttgagcgtcgatttttgtgatgctcgtcaggggggcggagcctatggaaaaacgccagcaacgcggcctttttacggttcctggccttttgctggccttttgctcacatgttctttcctgcgttatcccctgattctgtggataaccgtattaccgcctttgagtgagctgataccgctcgccgcagccgaacgaccgagcgcagcgagtcagtgagcgaggaagcggaagagcgcccaatacgcaaaccgcctctccccgcgcgttggccgattcattaatgcagctggcacgacaggtttcccgactggaaagcgggcagtgagcgcaacgcaattaatgtgagttagctcactcattaggcaccccaggctttacactttatgcttccggctcgtatgttgtgtggaattgtgagcggataacaatttcacacaggaaacagctatgacatgattacgccaagcttgcatgcctgcaggtcgactctagaggatccccgggtaccgagctcgaattcactggccgtcgttttacaacgtcgtgactgggaaaaccctggcgttacccaacttaatcgccttgcagcacatccccctttcgccagctggcgtaatagcgaagaggcccgcaccgatcgcccttcccaacagttgcgcagcctgaatggcgaatggcgataagctagcttcacgc

SEQ ID NO: 6 - DNA, 20 bp, synthetic construct
  source 1..20: mol_type = other DNA
gccgactgaaaggttcacgt

SEQ ID NO: 7 - DNA, 25 bp, synthetic construct
  source 1..25: mol_type = other DNA
tgaattccttagaatcagccagcac

SEQ ID NO: 8 - DNA, 25 bp, synthetic construct
  source 1..25: mol_type = other DNA
gtgctggctgattctaaggaattca

SEQ ID NO: 9 - DNA, 20 bp, synthetic construct
  source 1..20: mol_type = other DNA
tgagcagcaacgccaaggta